European Patent Specification EP 3 638 770 B1, published January 18, 2023. Title: RECOMBINANT YEAST CELL. Applicant: DSM IP ASSETS B.V. The sequence listing filed with the application follows.

SEQUENCE LISTING (4 sequences)

SEQ ID NO: 1 - protein, 459 aa, T. dinitrificans
  Amino acid sequence of T. denitrificans Rubisco large subunit CbbM
MDQSARYADLSLKEEDLIKGGRHILVAYKMKPKSGYGYLEAAAHFAAESSTGTNVEVSTTDDFTKGVDALVYYIDEASEDMRIAYPLELFDRNVTDGRFMLVSFLTLAIGNNQGMGDIEHAKMIDFYVPERCIQMFDGPATDISNLWRILGRPVVNGGYIAGTIIKPKLGLRPEPFAKAAYQFWLGGDFIKNDEPQGNQVFCPLKKVLPLVYDAMKRAQDDTGQAKLFSMNITADDHYEMCARADYALEVFGPDADKLAFLVDGYVGGPGMVTTARRQYPGQYLHYHRAGHGAVTSPSAKRGYTAFVLAKMSRLQGASGIHVGTMGYGKMEGEGDDKIIAYMIERDECQGPVYFQKWYGMKPTTPIISGGMNALRLPGFFENLGHGNVINTAGGGSYGHIDSPAAGAISLRQSYECWKQGADPIEFAKEHKEFARAFESFPKDADKLFPGWREKLGVHS

SEQ ID NO: 2 - protein, 352 aa, S. oleracea
  Amino acid sequence of S. oleracea phosphoribulokinase (prk)
MSQQQTIVIGLAADSGCGKSTFMRRLTSVFGGAAEPPKGGNPDSNTLISDTTTVICLDDFHSLDRNGRKVEKVTALDPKANDFDLMYEQVKALKEGKAVDKPIYNHVSGLLDPPELIQPPKILVIEGLHPMYDARVRELLDFSIYLDISNEVKFAWKIQRDMKERGHSLESIKASIESRKPDFDAYIDPQKQHADVVIEVLPTELIPDDDEGKVLRVRMIQKEGVKFFNPVYLFDEGSTISWIPCGRKLTCSYPGIKFSYGPDTFYGNEVTVVEMDGMFDRLDELIYVESHLSNLSTKFYGEVTQQMLKHQNFPGSNNGTGFFQTIIGLKIRDLFEQLVASRSTATATAAKA

SEQ ID NO: 3 - protein, 97 aa, E. coli [sequence omitted]

SEQ ID NO: 4 - protein, 548 aa, E. coli
  Amino acid sequence of E. coli groEL
MAAKDVKFGNDARVKMLRGVNVLADAVKVTLGPKGRNVVLDKSFGAPTITKDGVSVAREIELEDKFENMGAQMVKEVASKANDAAGDGTTTATVLAQAIITEGLKAVAAGMNPMDLKRGIDKAVTAAVEELKALSVPCSDSKAIAQVGTISANSDETVGKLIAEAMDKVGKEGVITVEDGTGLQDELDVVEGMQFDRGYLSPYFINKPETGAVELESPFILLADKKISNIREMLPVLEAVAKAGKPLLIIAEDVEGEALATLVVNTMRGIVKVAAVKAPGFGDRRKAMLQDIATLTGGTVISEEIGMELEKATLEDLGQAKRVVINKDTTTIIDGVGEEAAIQGRVAQIRQQIEEATSDYDREKLQERVAKLAGGVAVIKVGAATEVEMKEKKARVEDALHATRAAVEEGVVAGGGVALIRVASKLADLRGQNEDQNVGIKVALRAMEAPLRQIVLNCGEEPSVVANTVKGGDGNYGYNAATEEYGNMIDMGILDPTKVTRSALQYAASVAGLMITTECMVTDLPKNDAADLGAAGGMGGMGGMGGMM